European Patent Specification EP 3 875 103 B1, published June 25, 2025. Title: Peptide for promoting mucous membrane permeation and composition comprising the same. Applicant: Soonchunhyang University Industry Academy Cooperation Foundation. The sequence listing filed with the application follows.

SEQUENCE LISTING (15 sequences)

SEQ ID NO: 1 - protein, 6 aa, Artificial Sequence
  synthetic peptide
  PEPTIDE (2): Xaa is 3-Azidoalanine
FXIGRL

SEQ ID NO: 2 - protein, 6 aa, Artificial Sequence
  synthetic peptide
  PEPTIDE (1): Xaa can be Ala Val Leu Ile Pro Trp Tyr or Met
  PEPTIDE (2): Xaa is 3-Azidoalanine
XXIGRL

SEQ ID NO: 3 - protein, 6 aa, Artificial Sequence
  synthetic peptide
  PEPTIDE (2): Xaa is 3-Azidoalanine
  PEPTIDE (3): Xaa can be Ala Val Leu Pro Trp or Met
FXXGRL

SEQ ID NO: 4 - protein, 6 aa, Artificial Sequence
  synthetic peptide
  PEPTIDE (2): Xaa is 3-Azidoalanine
  PEPTIDE (4): Xaa can be Ser Thr Tyr Asn Ala or Gln
FXIXRL

SEQ ID NO: 5 - protein, 6 aa, Artificial Sequence
  synthetic peptide
  PEPTIDE (2): Xaa is 3-Azidoalanine
  PEPTIDE (5): Xaa can be Lys or His
FXIGXL

SEQ ID NO: 6 - protein, 6 aa, Artificial Sequence
  synthetic peptide
FCIGRL

SEQ ID NO: 7 - protein, 6 aa, Artificial Sequence
  synthetic peptide
  PEPTIDE (1): Xaa can be Ala Val Leu Ile Pro Trp Tyr or Met
XCIGRL

SEQ ID NO: 8 - protein, 6 aa, Artificial Sequence
  synthetic peptide
  PEPTIDE (2): Xaa can be Gly Ser Thr Tyr Asn or Gln
FXIGRL

SEQ ID NO: 9 - protein, 6 aa, Artificial Sequence
  synthetic peptide
  PEPTIDE (3): Xaa can be Ala Val Leu Pro Trp or Met
FCXGRL

SEQ ID NO: 10 - protein, 6 aa, Artificial Sequence
  synthetic peptide
  PEPTIDE (4): Xaa can be Ser Thr Tyr Asn Ala or Gln
FCIXRL

SEQ ID NO: 11 - protein, 6 aa, Artificial Sequence
  synthetic peptide
  PEPTIDE (5): Xaa can be Lys or His
FCIGXL

SEQ ID NO: 12 - protein, 6 aa, Artificial Sequence
  synthetic peptide
  PEPTIDE (2): Xaa is 3-Azidoalanine
  PEPTIDE (6): Xaa is a variant of leucine wherein the carboxyl group -COOH is modified to -CONH2
FXIGRX

SEQ ID NO: 13 - protein, 6 aa, Artificial Sequence
  synthetic peptide
  PEPTIDE (6): Xaa is a variant of leucine wherein the carboxyl group -COOH is modified to -CONH2
FCIGRX

SEQ ID NO: 14 - protein, 7 aa, Artificial Sequence
  synthetic peptide
  PEPTIDE (1): Xaa is 3-Azidoalanine
XFCIGRL

SEQ ID NO: 15 - protein, 7 aa, Artificial Sequence
  synthetic peptide
  PEPTIDE (1): Xaa is 3-Azidoalanine
  PEPTIDE (7): Xaa is a variant of leucine wherein the carboxyl group -COOH is modified to -CONH2
XFCIGRX